European Patent Application EP 4 710 932 A1, published March 18, 2026. Title: Composition for the treatment of a disease linked to aberrant endoplasmic reticulum and mitochondria connections. Applicant: Administración General de la Comunidad Autónoma de Euskadi. The sequence listing filed with the application follows.

SEQUENCE LISTING (4 sequences)

SEQ ID NO: 1 - DNA, 20 bp, synthetic construct
  source 1..20: mol_type = other DNA
cacccaagaacagggtttgt

SEQ ID NO: 2 - DNA, 20 bp, synthetic construct
  source 1..20: mol_type = other DNA
tggccatgggtatgttgtta

SEQ ID NO: 3 - DNA, 25 bp, synthetic construct
  source 1..25: mol_type = other DNA
tgctgtctccatgtttgatgtatct

SEQ ID NO: 4 - DNA, 22 bp, synthetic construct
  source 1..22: mol_type = other DNA
tctctgctccccacctctaagt